European Patent Application EP 4 299 766 A2, published January 3, 2024. Title: Method for producing artificial recombinant rotavirus. Applicant: Osaka University. The sequence listing filed with the application follows.

SEQUENCE LISTING (33 sequences)

SEQ ID NO: 1 - DNA, 3854 bp, Mammalian orthoreovirus
  source 1..3854: mol_type = other DNA
gctacacgttccacgacaatgtcatccatgatactgactcagtttggaccgttcattgagagcatttcaggtatcactgatcaatcgaatgacgtgtttgaagatgcagcaaaagcattctctatgtttactcgcagcgatgtctacaaggcgctggatgaaatacctttctctgatgatgcgatgcttccaatccctccaactatatatacgaaaccatctcacgattcatattattacattgatgctctaaaccgtgtgcgtcgcaaaacatatcagggccctgatgacgtgtacgtacctaattgttctattgttgaattgctggagccacatgagactctgacatcttatgggcggttgtccgaggccatcgagaatcgtgccaaggatggggacagccaagccagaatcgccacaacgtatggtagaatcgctgaatctcaagctcgacagattaaggctccattggagaagtttgtgttggcactattagtggccgaagcaggggggtctttatatgatccagttttgcagaagtatgatgagattccagatctatcgcataattgccctttatggtgttttagagagatctgtcgtcacatatctggtccattaccagatcgggcaccttatctttacttatctgcaggggtattctggttaatgtcaccacgaatgacgtctgcaatccctccgctactatccgatcttgttaatttagctattttgcaacaaactgcgggtttagatccatcattagtgaaattgggagtacagatatgccttcatgcagcagctagctcaagttattcatggtttatcttaaagactaagtctatttttcctcaaaacacgttgcacagtatgtatgaatctctagaagggggatactgtcctaatcttgaatggttagagcctagatcagactataagttcatgtacatgggagtcatgccattgtccgctaagtatgctaggtcggcgccgtccaatgataagaaagcgcgggaacttggcgagaaatatggactgagctcagtcgtcggtgagcttcgtaaacggacaaagacgtatgttaaacatgactttgcttcagtgaggtacattcgtgacgctatggcatgtactagcggtattttcttggtaagaacacccaccgaaacggtattgcaagaatatacgcagagtccggagattaaggttcccattccccagaaagactggacaggcccaataggtgaaatcagaattctaaaagatacaacaagttccatcgcgcgttacttatatagaacatggtacttggcagcggcgagaatggcggctcaaccacgtacgtgggatccattgtttcaagcgattatgagatctcaatacgtgacagctaggggtggatctggcgcagcactccgcgaatctttgtatgcaatcaatgtgtcgttacctgatttcaagggcttaccagtgaaggcagcaactaagatattccaggcggcacaattagcgaacttgccgttctcccacacatcagtggctatactagctgacacttcaatgggattgcgaaatcaggtgcagaggcggccacgatccattatgccattaaatgtgccccagcagcaggtttcggcgccccatacattgacagcggattacattaactaccacatgaatctatcacccacgtctggtagtgcggtcattgagaaggtgattcctttaggtgtatacgcttcgagccctcctaaccagtcgatcaacattgacatatctgcgtgtgacgctagtattacttgggatttctttctgtcagtgattatggcggctatacacgaaggtgtcgctagtagctccattggaaaaccatttatgggggttcctgcatccattgtaaatgatgagtctgtcgttggagtgagagctgctaggccgatatcgggaatgcagaacatgattcagcatctatcgaaactatataaacgtggattttcatatagagtaaacgattctttttctccaggtaacgattttactcatatgactaccactttcccgtcaggttcaacagccacctctactgagcatactgctaataatagtacgatgatggaaactttcctgacagtatggggacccgaacatactgacgaccctgacgtcttacgtttaatgaagtctttaactattcaaaggaattacgtatgtcaaggtgatgatggattaatgattatcgatgggactactgctggtaaggtgaacagtgaaactattcagaacgatctagaattaatctcaaaatatggtgaggaattcggatggaaatatgacatagcgtacgatgggactgccgaatacttaaagctatacttcatatttggctgtcgaattccaaatcttagtcgccatccaatcgtggggaaagaacgggcgaattcttcagcagaggagccatggccagcaattctagatcagattatgggtgtcttctttaatggtgttcatgatgggttacagtggcagcggtggatacgttattcatgggctctatgctgtgctttctcacgtcaaagaacaatgattggtgagagcgtgggttaccttcaatatcctatgtggtcttttgtctactggggattaccactggttaaagcgtttgggtcagacccatggatattttcttggtacatgcctactggagatctgggaatgtatagttggattagcttgatacgccctctgatgacaagatggatggtggctaatggttacgtaactgacagatgctcaaccgtattcgggaacgcagattatcgcaggtgtttcaatgaacttaaactatatcaaggttattatatggcacaattgcccaggaatcctaagaagtctggacgagcggcctctcgggaggtaagagaacaattcactcaggcattatccgactatctaatgcaaaatccagagctgaagtcacgtgtgctacgtggtcgtagtgagtgggagaaatatggagcggggataattcacaatcctccgtcattattcgatgtgccccataaatggtatcagggtgcgcaagaggcagcaatcgctacgagagaagagctggcagaaatggatgagacattaatgcgcgctcgaaggcacagctattcgagcttttcaaagttattagaggcgtatctgctcgtgaaatggcgaatgtgcgaggcccgcgaaccgtcggttgatttgcgattaccattatgtgcgggtattgacccattaaactcagatccttttctcaagatggtaagcgttggaccaatgctccagagtacgagaaagtactttgctcagacactattcatggcaaagacggtgtcgggtcttgacgttaacgcgattgatagcgcgttattacgactgcgaacattaggtgctgataagaaagcattaacggcgcagttattaatggtggggcttcaggagtcagaagcggacgcattggccgggaagataatgctacaggatgtgaatactgtgcaattagccagagtggttaacttagctgtgccagatacttggatgtcgttagactttgactctatgttcaaacaccacgtcaagctgcttcccaaagatggacgtcatctaaatactgatattcctcctcgaatgggatggttacgggccattttacgattcttaggtgccggaatggtaatgactgcgactggagttgctgtcgacatctatctggaggatatacatggcggtggtcggtcacttggacagagattcatgacttggatgcgacaggaaggacggtcagcgtgagtctaccatgggtcgtggtgcgtcaactcatc

SEQ ID NO: 2 - DNA, 3915 bp, Mammalian orthoreovirus
  source 1..3915: mol_type = other DNA
gctattggcgcaatggcgaacgtttggggagtgagacttgcagactctttatcatcacccactattgagacaagaactcgtcattacacactacgcgatttctgttccgacctggatgctgtggctggcaaggaaccctggagacctttgcgcaatcagagaacgaatgacattgtcgccgttcaattgtttaggccactgcagggattggtgcttgacacgcagttctatggattccctggcattttctcagaatgggagcagtttataaaggaaaaactccgcgtattaaaatatgaggttttgcggatctacccaatcagtaattataatcatgaacgtgtcaatgtcttcgtagcaaatgctcttgtcggtgcgttcctatccaaccaagccttctatgacctgttgcctctattagtaataaatgataccatgataaatgacttacttgggacaggtgccgccctttctcaattttttcaatcccatggtgaggttttagaagttgccgcaggaaggaagtacctgcaaatgaagaactactcgaacgatgacgatgatccacctttgttcgctaaagatctgtcggactatgcgaaggcgttttacagtgacacgtttgagactctagaccgatttttctggacacatgactcatctgcgggcgtcctagtgcactatgataagcccactaacgggaatcattacatcttgggtactctgacgcagatggttagtgcgcctccgcatatcattaacgctactgacgcattgttgctcgaatcgtgcttagaacaatttgcggcgaatgtgagagccaggccagcgcagcctgttgcgagattggatcaatgttatcatttacggtggggtgctcaatatgttggcgaggactcattgacgtaccgtttgggggtactttcgctgctggctaccaacggatatcaattagctagaccgatccctaagcaattgacgaatcgatggctctctagttttgtcagtcaggtaatgtcggatggtgtaaatgagacgccattatggcctcaagagagatatgtccaaatagcctacgattcaccatctgtagtcgatggagccacgcactatggctatgttaggcgaaatcagttgcggttgggcatgagggtgtccgctcttcagtcattgagtgatactccggctccgatacagtggttaccgcagtatactattgaacaggcagctgttgatgagggagatctaatggtttctcgcttgactcaactaccattacgtcctgactatggcagcatatgggttggtgatgccctatcgtattatgttgattacaatcgcagccatagagttgtactatcatccgaactaccacagctaccagatacatactttgacggagatgagcaatacggtcgtagcttgttctctctagcacgaaaaattggtgatcgatctctcatcaaagatacagcagtgcttaagcatgcgtaccaggccattgatccaaacactggaaaggaataccttcgcgcaggacagtccgttgcatactttggggcatcagctggtcattcaggggcggatcagcctctagtaattgagccatggacgcagggtaagattagtggtgtgcctccgccctcctcagttagacagtttgggtatgatgttgctaaaggtgcgatcgtagacttagcaagaccgttcccgtcgggcgactaccaatttgtatattctgacgtcgatcaggtcgttgatggccacgatgatctcagcatatcctcaggactggtggagagtctattagactcatgcatgcatgccacatccccaggtgggtcattcgtgatgaagatcaacttcccgacacgcactgtctggcactatatagagcagaagattctcccaaatattacctcgtacatgttgattaaaccattcgtgactaataatgtagagttattctttgtggcttttggtgtgcatcaacaatcagcattgacatggacgtctggggtgtatttcttcctggtcgatcacttctatcgatacgagacattgtctacgatttcacgtcagttgccatcgttcggatacgttgatgatgggtcgtctgtgacaggcattgagatgatcagtcttgaaaatccaggcttttcaaacatgacccaagctgcacgtgttgggatatcagggttgtgtgcgaatgtcggtaatgcgcgtaaattaatatctattcatgaatcccatggggcacgcgtgctcaccatcacatcaagaagatctccagcttcggccaggcggaaagctcgcttacgctatttgccactcgtagacccacgatctttggaagtgcaggcacgtacgatactgccatctaacccagtgttgtttgataacgtaaacggagcatcgcctcacgtatgtttgacgatgatgtataactttgaagtgtctagtgcggtgtatgatggtgatgtagtacttgatcttggtaccggtcctgaagcgaagattctggagctgattcctccaacatccccggtaacatgcgtagacattaggccaacggcacagccgagtggctgttggaacgtacgtacgacttttctagagcttgattacttaagtgacggttggataacgggtatacgtggcgacatcgtcacttgcatgctgtctctgggtgctgctgctgctggaaaatccatgacgttcgacgcggcattccaacagctagtgaaagttcttactaaaagtacagctaacgtgttgttgattcaagtcaactgcccaacggatgtgatccgaacaattaagggatatttggagatagatcaaactaataagcggtacagatttccaaagtttggccgcgatgaaccgtactctgacatggattcattagagcgcatatgtcgggctgcatggccaaattgttccatcacgtgggtgcccttgtcctatgacctgcgttggactaagcttgctctacttgaatcgactacactgagcagtgcatcagtgagaattgctgaattgatgtacaagtacatgcccgttatgaggatagatattcatgggttacccatggaaaagcaaggcaatttcatagtgggtcagaactgctctttgactataccgggcttcaacgcacaggacgtattcaattgttacttcaactccgcgctcgccttctctactgaggatgttaattctgcaatgataccacaggtgacggctcagtttgatgctaacaaaggagagtggtcattggacatggtgttctcagacgctggtatctacacaatgcaggcattggtcggttccaacgcaaatcctgtgtctctgggttcgtttgtagtggactctccggatgtggacataacagatgcatggcctgctcagctggactttaccatagctggcactgacgtcgacattacagttaatccttattaccgcttgatggcctttgtgaggattgatggacaatggcagattgcgaatcctgataaattccaatttttctcatcaagtacaggaacgttagtgatgaatgtaaagttagatatagctgataggtacttgttatactacattcgtgacgttcaatctagggatgtgggattttacatacagcacccattacagttattaaatactattacgctgcctacaaatgaggacttattcttgagcgctcctgacatgcgcgagtgggcagtaaaggagagtggtaataccatatgcatacttaatagtcaaggttttgtgccacctcaggattgggatgttcttaccgatactattagctggtctccttcgctcccaacttatgtggtgcctccgggtgattatactctgacacctctgtaactcattacccctcgtgagcgtgcctaattcatc

SEQ ID NO: 3 - DNA, 3901 bp, Mammalian orthoreovirus
  source 1..3901: mol_type = other DNA
gctaatcgtcaggatgaagcggattccaaggaagacaaagggcaaatccagcggaaagggcaatgactcaacagaaagatcggacgatggctcgagccaattacgagacaagcaaaacaataaggctggccctgccactacggagcctggcacatctaaccgagagcaatacagagcccgaccaggtattgcatctgtgcagagggccactgaaagtgcagaactgcccatgaagaataatgacgaagggacgccagataagaaaggaaatactaggggcgacttagttaatgagcatagtgaggctaaagacgaggcggatgaagcgacgcagaagcaggcaaaagacacagacaaaagtaaagcgcaagtcacatattcagacactggtatcaataatgctaatgaactgtcaagatctgggaatgtggataatgagggtggaagtaatcagaagccgatgtccaccagaatagctgaagcaacgtctgctatagtgtcgaaacatcctgcgcgtgttgggttaccacctaccgctagcagtggtcatgggtatcagtgccacgtctgttctgcagtcctgtttagtcctttagacctagatgcccacgtcgcctcacatggtttgcatggtaacatgacattaacatcgagtgagattcagcgacatataactgagttcatcagctcatggcaaaatcatcctattgttcaagtttcggctgatgtcgaaaataagaagactgctcaactgcttcacgctgacactcctcgactcgtcacttgggatgctggtttgtgtacttcgttcaaaatcgtcccgattgtgccagctcaggtgccgcaggatgtactggcctatacgtttttcacctcttcatatgccatccaatcaccgtttccagaggcggcagtgtctaggattgtggtgcatacgagatgggcatctaatgttgactttgaccgagattcgtctgtcatcatggcgccacctacagaaaacaatatccatttgtttaagcagttactaaatactgaaaccctgtctgtaaggggggctaatccgctaatgtttagagcgaacgtgttgcatatgttgctggagttcgtattagataacttgtatctgaacagacatacgggattctctcaagaccacacaccatttactgagggtgctaatctgcgctcacttcctggccccgatgctgagaaatggtactcgattatgtatccaacgcgcatgggaacgccgaatgtatcaaaaatatgtaatttcgtcgcctcttgtgtgcgaaatcgggttggacgatttgatcgagcacagatgatgaacggagctatgtcagagtgggtggatgtcttcgagacttcagacgcgcttaccgtctccattcgaggtcgatggatggctagactagctcgcatgaacataaatccaacagagatcgaatgggcgttgactgaatgtgcacaaggatatgtgactgtcacaagtccttacgctcctagcgtaaatagattgatgccctatcgtatctccaacgctgagcggcaaatatcacagataatcaggatcatgaacattggcaataacgcgacggtgatacaacctgttctgcaagatatttcagtactccttcaacgcatatcaccactccaaatagatccaactattatttccaacactatgtcaacagtctcggagtctactactcagaccctcagccccgcgtcctcaattttgggtaaactacgaccgagtaactcagatttctctagttttagagtcgcgttggctggatggctttataatggagttgtgacgacggtgattgatgatagttcatatccaaaagacggtggcagcgtgacctcacttgaaaatctgtgggatttcttcatccttgcgcttgctctaccactgacaactgacccctgtgcacctgtgaaagcattcatgaccttagctaacatgatggttggtttcgagacaatccctatggataatcagatctatactcaatcgagacgcgcgagtgctttctcaacgcctcacacgtggccacgatgcttcatgaatatccagttaatttctccaatcgatgctcctatcttgcgacagtgggctgaaattattcatagatactggcctaacccttcacagattcgttatggtgcaccgaacgttttcggctcggcaaatttgttcactccacctgaggtgctgttattgccaatcgatcatcaaccagctaatgtaacaacgccaacgctggacttcaccaatgagttgactaattggcgcgctcgtgtctgtgagcttatgaagaatcttgttgataatcaaagatatcaacctggatggacacaaagtctagtctcgtcaatgcgcggaacgctagacaaattgaagttgattaaatcgatgacacccatgtatctgcaacagctggctccggtagagttagcagtgatagctcccatgttgcctttcccacctttccaggtgccctacgtccgtctcgatcgtgatagagttccaacaatggtcggagtaacacgacagtcacgagatactattactcagccagcgctatcgctgtcgacgaccaatactactgttggcgtgccactagctctagacgcgagggctatcaccgttgcgctgttgtcagggaaatatccgccggatttagtgacaaatgtatggtacgctgatgccatttatccaatgtatgcagacactgaggtgttctctaatcttcagagagacatgattacctgcgaggccgtgcagacattagtgactctggtggcgcaaatatcagagacccagtatcctgtagataggtatcttgattggatcccatcactgagagcatcggcggcgacggcggcgacatttgctgagtgggttaatacttcaatgaagacggcgtttgatttgtctgacatgctgttagagcctctcctaagcggtgatccgaggatgactcaactagcgattcagtatcagcaatacaatggcagaacgtttaatgtcatacctgaaatgccaggttcagttattgctgactgcgttcaactaacagcagaagtcttcaatcacgaatataacctgtttgggattgcgcggggtgatatcatcattggccgtgttcagtcgacacatttgtggtcaccgctggctcctccacctgacctggtgtttgatcgtgacactcctggtgttcacatcttcggacgagattgccgcatatcgtttggaatgaatggcgccgcgccaatgattagagatgagactggaatgatggtgccttttgaaggaaattggatcttcccactggcgctttggcaaatgaatacacgatattttaatcaacaattcgacgcgtggattaagacaggagagttgcgaatccgtattgagatgggcgcgtatccatatatgttgcattactatgatccacgtcagtacgctaatgcatggaatttaacatccgcctggcttgaagaaattacaccgacgagcatcccatccgtgcctttcatggtgcccatttcaagtgatcatgacatttcctctgccccagctgtccaatacatcatctcgactgaatataatgatcggtctttattctgcactaactcatcatctccccaaactatcgctggaccagacaaacacattccagttgaaagatataacattctgaccaaccccgacgctccacccacgcagatacaactgcctgaagttgttgacttgtataacgtcgtcacacgctatgcgtatgagactccgcctattaccgctgtcgttatgggtgttccttgatcctcatcctcccaacaggtgctagagcatcgcgctcgatgctagttgggccgattcatc

SEQ ID NO: 4 - DNA, 2304 bp, Mammalian orthoreovirus
  source 1..2304: mol_type = other DNA
gctattcgcggtcatggcttacatcgcagttcctgcggtggtggattcacgttcaagtgaggctattggactgctagaatcgtttggagtagacgctggggctgatgcgaatgacgtttcatatcaagatcatgactatgtgttggatcagttacagtatatgttagatggatatgaggctggcgacgttatcgatgcactcgtccacaagaattggttacatcactctgtctattgcttgttgccacccaaaagtcaactactagagtattggaaaagtaatccttcagtgataccggacaacgttgatcgtcggcttcgtaaacgactaatgctaaagaaagatctcagaaaagatgatgaatacaatcaactagcgcgtgctttcaagatatcggatgtctacgcacctctcatctcatccacgacgtcaccgatgacaatgatccagaacttgaatcaaggcgagatcgtgtacaccacgacggacagggtaattggggctagaatcttgttatatgctcctagaaagtactatgcgtcaactctatcatttactatgactaagtgcatcattccgtttggcaaagaggtgggtcgtgttcctcactctagatttaatgttggcacatttccatcaattgctaccccgaaatgttttgtcatgagtggggttgatattgagtccatcccaaatgaattcatcaagttgttttaccagcgcgtcaagagtgttcacgccaatatactaaatgacatatcacctcagatcgtctctgacatgataaacagaaagcgtttgcgcgttcatactccatcagatcgtcgagccgcgcagttgatgcatttgccctaccatgttaaacgaggagcgtctcacgtcgacgtttacaaggtggatgttgtagacgtgttgttcgaggtagtggatgtggccgatgggttgcgcaacgtatctaggaaactaactatgcataccgttccggtatgtattcttgaaatgttgggtattgagattgcggactattgcattcgtcaagaggatggaatgttcacagattggttcctacttttaaccatgctatctgatggcttaactgatagaaggacgcattgtcaatacttgattaatccgtcaagtgtgcctcctgatgtgatacttaacatctcaattactggatttataaataggcatacaatcgatgtcatgcctgatatatatgacttcgttaaacccattggcgctgtgctgcctaagggatcatttaaatcaacaattatgagagttcttgattcaatatcaatattaggagtccagatcatgccgcgcgcgcatgtagttgactcggatgaggtgggcgagcaaatggagcctacgtttgagcatgcggttatggagatatacaaagggattgctggcgttgactcgctggatgatctcatcaagtgggtgctgaactcggatctcattccgcatgatgacaggcttggccaattatttcaagcgtttctgcctctcgcaaaggacttgttagctccaatggccagaaagttttatgataactcaatgagtgagggtagattgctgacattcgctcatgccgacagtgagttgctgaacgcaaattactttggtcatttattgcgactaaaaataccatatattacagaggttaatctgatgattcgcaagaatcgtgagggtggagagctatttcagcttgtgttatcgtatctatataaaatgtatgctactagcgcgcagcctaaatggtttggatcattattgcgattgttaatatgtccctggttacatatggagaaattaataggagaagcagacccggcatctacgtcggctgaaattggatggcatatccctcgtgaacagctgatgcaagatggatggtgtggatgtgaagatggattcattccctatgttagcatacgtgcgccaagactggttatggaggagttgatggagaagaactggggccaatatcatgcccaagttattgtcactgatcagcttgtcgtaggcgaaccgcggagggtatctgccaaggctgtgatcaagggtaatcacttaccagttaagttagtttcacgatttgcatgtttcacattgacggcgaagtatgagatgaggctctcgtgcggccatagcactggacggggggctgcatacaatgcgagactagctttccgatctgacttggcgtgatccgtgacatgcgtagtgtgacacctgcccctaggtcaatgggggtagggggcgggctaagactacgtacgcgcttcatc

SEQ ID NO: 5 - DNA, 2203 bp, Mammalian orthoreovirus
  source 1..2203: mol_type = other DNA
gctaatctgctgaccgtcactctgcaaagatggggaacgcttcctctatcgttcagacgatcaacgttactggagatggcaatgtattcaaaccctcagctgagacttcatccaccgctgtaccgtcactgagtctatcacctggaatgttaaatcctggaggagtaccatggattgcgattggagatgaaacatccgttacttcaccgggtgcattgcggcgaatgacttcgaaggatatcccagagacagcaataatcaatacggataattcatcaggcgcggtgccaagtgaatcagcattagtgccctataatgatgagccattggtagtggtgacggagcacgctatcgcaaacttcaccaaagccgagatggcacttgagttcaatcgtgagttcctcgataaattgcgcgtgctgtcagtgtcaccaaaatattccgaccttctgacgtatgttgattgttacgttggtgtgtcggcccgtcaggccctaaataatttccagaagcaggtgcctgtgattacacctactagacaaacaatgtatgttgactccatacaggcggccttgaaagccttagagaaatgggaaattgatttgagagtggctcagacactgttgcctacaaatgtcccaattggggaggtctcttgtccaatgcagtcagtagtgaaactattagacgatcagctgccggacgatagccttatacggaggtatcctaaggaggccgctgttgctttggctaaaaggaatggagggatacagtggatggacgtatcagaaggaactgtgatgaatgaggccgtgaatgctgtcgcagcaagtgccctggcaccttccgcatcagccccacccttagaagagaaatcgaaattgactgagcaagcgatggatcttgtaactgcagctgaacctgagataatcgcatctctcgtaccagttccagcgcccgtgtttgccattccacctaagccagccgactataatgtgcgtactttgaagatcgatgaggccacatggttacgaatgatcccaaaaactatgggtacgccttttcaaatccaagtgactgacaacacaggaactaactggcaccttaacttgagaggagggacacgcgtagtgaacttggatcagattgctccgatgagattcgttctggatctggggggaaaaagctataaggagacaagttgggatccaaatggtaagaaggttgggtttatcgtatttcaatctaagattccttttgagctttggaccgccgcctcacagattggccaagctacagtggttaactatgttcagctatatgctgaagacagctcatttaccgcccagtccatcatcgccactacatcgttggcttataattatgaacctgagcaattgaataagactgaccctgagatgaactattaccttttagcgactttcatagactcagctgctataacaccgacaaacatgacacagcctgatgtttgggatgctctgttgacgatgtctccactgtccgctggagaggtgactgtgaagggtgcggtagtaagcgaggtggtcccagcggagttgatagggagctatactccagagtcactaaatgcctcacttccgaatgacgctgctagatgtatgatcgatagagcttcgaagatagccgaggctataaaaattgatgatgacgccgggccagacgaatactctcccaactctgtaccgatccaaggtcagcttgctatttctcaacttgagactgggtatggtgtacggatattcaatcccaaaggaattctctcaaaaatcgcatctagagctatgcaggcttttattggtgatccaagtacaattattacgcaggcagcaccggtgctgtcagataagaataattggattgcattggcacaaggagttaagactagtttgcgtactaaaagtttatcggcgggggtgaagacggcggtgagtaagctgagctcatccgagtctattcaaaattggactcaaggattcttggataaggtatcgacgcactttccagcgcctaagcccgactgtccgaccaacggagatggcagtgaaccgtctgctcggcgagtgaagcgcgactcatacgcaggagtggttaagcgtgggtatacacgctaagctgctcgccctggtgacacggggttaagggatgcaggcacatcatc

SEQ ID NO: 6 - DNA, 2241 bp, Mammalian orthoreovirus
  source 1..2241: mol_type = other DNA
gctaaagtgaccgtggtcatggcttcattcaagggattctccgtcaacactgttccagtttccaaggccaaacgtgatatatcatctcttgccgctactcctggaattcgctcacaacccttcactccgtctgtagacatgtctcaatcgcgtgaattccttacaaaggcaattgagcaagggtctatgtctataccttatcagcatgtgaatgttccaaaagttgatcgtaaggttgttagtttggtagtgcgaccgttttcttcaggtgctttttctatctctggagtgatttcaccggcgcacgcttatctattggattgtctacctcagcttgaacaggcgatggcgtttgttgcttcacctgaatctttccaggcttctgatgtcgcaaaacgctttgctataaagccgggcatgagccttcaggatgccatcactgccttcatcaactttgtgtccgcgatgctgaaaatgacggtgactcgtcaaaattttgatgtcatcgtggctgagatcgagaggcttgcttcaaccagcgtatctgtccgaactgaagaggcaaaggttgccgatgaagagctgatgctgttcgggctagatcatagagggccacagcagcttgatatttctaatgctaaagggataatgaaagctgcagatattcaggcaactcatgacgttcatttggcaccaggcgtcggtaatatcgatcctgagatctacaatgagggacggttcatgtttatgcagcacaaaccactcgcggcagatcagtcgtatttcacgttggagactgcggattatttcaagatctacccaacatatgatgagcatgatagcagaatggctgatcagaagcagtcagggttgatattgtgcactaaagatgaggtgttggctgagcaaactatttttaagctagatgcccctgatgataaaaccgttcatctattggatcgcgacgacgatcacgttgttgctagatttactaaggtgtttatagaagatgtggcccccgggcatcatgctgcgcaaaggtctggccaacgctctgtgcttgatgacctatatgccaacacccaagtggtttcaatcacttctgctgctctgaagtgggtagttaaacacggtgtgtccgacgggattgtgaatagaaagaatgtcaaagtgtgtgttggttttgaccctttgtacactctatctacgcataatggagtgtctttgtgcgccctgctgatggatgaaaaactttccgtgctgaacagcgcatgtcgtatgacgctgcgttcactaatgaaaactggacgtgatgctgatgcacatagggcttttcagcgagtgctctctcagggatacgcatcattaatgtgctattatcacccttcacggaagttagcatatggtgaggtgctttttctagagcgatccagtgacatggtagacgggattaaactacagttggacgcatctagacagtgtcatgagtgtcccgtgttgcagcagaaagtagttgagttggaaaaacagattatcatgcagaagtccattcagtcagatcctaccccaatggcgctgcaaccactgttatctcagttgcgtgaactgtctagtgaggtcacccgactccagatggagttaagtcggactcagtccctgaatgctcagttggaagcggatgctaagtcagctcaagcatgtagtctggatatgtatttgagacaccacacctgcattaatggtcatacaaaagaagatgaactgcttgatgctgtacgtgtcgctccagatgtgaggaaagaaatcatggaaaagaggggcgaagtgagaaggggctggtgcgaacgtatctctaaggaagcggctgccaaatgccaaactgttattgatgacttgactcagatgaatggaaagcaggcacgagagataacagaattacgcgagtcagccgagaattatgagaagcagattgcggaattggtgggcactattactcaaaaccagatgacgtatcagcaagagctacaagctttggtagcgaagaatgtggaactggatacgatgaaccaacgtcaggctaaatcattgcgtattactccctcccttctatcagccactcctatcgattcagtcgacggcgctgctgacctgattgatttctccgttccaactgatgagctgtaaatgagctgtgacgcagtgttgccctaatcccttaagccttcccgacccctattcatc

SEQ ID NO: 7 - DNA, 1463 bp, Mammalian orthoreovirus
  source 1..1463: mol_type = other DNA
gctattcgcgcctatggatgcatctctcattacagagatacggaaaatagtactccaactatctgtatcaagcaatggctcccagtcaaaagaaatcgaggaaatcaagaaacaagtccaggtcaacgttgatgatatcagggctgccaatattaaactcgacggacttggaagacagattgctgacatcagcaatagcatctcaaccattgagtcaagattgggtgagatggataatcgacttgtgggtatctcgagtcaggtcacgcaattatctaactcagttagccagaacactcagagcatatcctcattgggtgacagaatcaatgctgtcgaaccacgagttgacagtctggatacggtcacgtctaatctcactggacgaacatccactttggaggcagatgttggaagcttacggacagaactagcagcgctaacaacacgggtgacaactgaggttacaaggttagatggtctaatcaatagtggccagaattcgattggtgagctatccacaagactatccaatgtggagacgtctatggtgacgacggctggacggggactgcagaaaaacggaaacaccttgaacgtcattgtaggtaatggaatgtggtttaatagttctaatcaattgcagctcgacctttcggggcaatcaaaaggggtgggatttgtcggcacaggaatggtggttaagattgatactaattattttgcttacaatagtaatggagagattacattggtgagtcaaatcaatgaattgccatcgcgcgtatcaacactggaatcagcgaaaatcgattcagttttacctccattaaccgtacgcgaagcgagcggcgtacgtaccctgagctttggttatgatacgagcgattttacaatcatcaactccgtactgtcgttacggtcacgtttgactcttccgacatacaggtaccctctggagctcgacacagcaaataatagagtgcaggtggcagatcgttttggcatgcgcacgggtacttggacgggacaattgcaatatcagcacccacaattgagttggagagcaaatgtcactttgaatttgatgaaggtggatgattggttggtgttgagcttttctcagatgacgactaactcaataatggcagatgggaaatttgtgattaattttgtgtctgggttatcttctggatggcagacgggggatactgaaccatcgtcaactattgatccattgtctacgacatttgccgcggtccaatttctaaataacggtcaacgcattgatgcgtttaggatcatgggagtatcggaatggacggatggagaattagagattaagaattatggtggcacatacaccggtcatactcaagtatattgggctccgtggacgatcatgtatccatgcaatgtgaggtgaatctagcgcgaaccctcggcacaaggggtcaatcatc

SEQ ID NO: 8 - DNA, 1331 bp, Mammalian orthoreovirus
  source 1..1331: mol_type = other DNA
gctattcgctggtcagttatggctcgcgctgcgttcctattcaagactgttggatttggtggtctgcaaaatgtgccaattaatgatgagttatcgtcacatctacttcgagccggtaattcgccatggcagctgactcagttcttagattggataagtcttggaagaggattagctacatcagctcttgttccaaccgctggttcaagatattatcagatgagttgtttattgagtggtaccctccagattccatttcgtcctaatcatcgatggggagatattaggtttctgcgtctagtgtggtcagctcctacgcttgacgggttggttgttgccccaccgcaggtcttagctcagccagcgttacaggcgcaggcagatcgagtgtatgattgtgatgattacccattcttagcacgtgacccgagatttaagcatcgagtgtatcaacaattgagcgccgtaactctgcttaacttgacggggtttggtccaatttcctatgttcgagtagacgaggatatgtggagtggggatgtgaaccagcttctcatgaactacttcgggcatacgtttgcggaaattgcgtatacattatgtcaagcttcagccaatagaccttgggagcatgatggtacgtatgcgaggatgactcaaattatactgtccttattttggttatcatatgtcggtgtaattcatcagcagaacacgtaccggacgttctatttccaatgcaatcggcgcggtgatgctgctgaagtatggattctttcctgctcattaaaccactccgcccagattagaccgggtaatcgcagtctattcgtcatgccaacaagtccagattggaatatggacgtcaatttgattttaagttcgacgttgacagggtgcttgtgttcgggctctcagttaccgcttattgacaataactcagtgcctgcggtttcgcgtaacatccatggttggactggcagagctggcaaccagctgcatggtttccaagtgcgacgaatggtgactgaattctgtgacagattaagacgcgatggagttatgactcaagctcagcaaaatcaaattgaagcgttggcagatcaaactcaacagtttaagagggataaacttgaggcgtgggctagggaagatgatcagtataatcaggctaatccgaattctacgatgttccgtacgaagccatttacgaatgcgcaatggggacgaggaaataccggagcgactagtgccgcaattgcagcccttatctaatcgtcttggagtgaggggatccccccacacccctcacgactgaccacacattcatc

SEQ ID NO: 9 - DNA, 1198 bp, Mammalian orthoreovirus
  source 1..1198: mol_type = other DNA
gctaaagtcacgcctgttgtcgtcactatggcttcctcactcagggctgcgatctctaagatcaagagagatgatgttggtcagcaagtttgtccaaattatgtcatgcttagatcatcggtcacaacgaaggtggtacgaaacgttgttgagtatcaaatccgtacaggtggattcttttcgtgcctagctatgttgagaccgctccagtatgctaaacgtgagcgtctgcttggacaaaggaatctggaacgcatatcgactagggacattcttcagacacgcgatttgcactcattgtgcatgccaactcctgacgcgccaatgtccaatcatcaggcagccaccatgagagagctgatctgcagctacttcaaggtcgaccacactgatgggttgaaatatatacccatggatgagagatattctccatcatcgcttgccagattgttcactatgggtatggctggactacacattaccactgagccttcctacaaacgtgtgcccatcatgcacttggcagcagatttggactgcatgacgttagctttaccctacatgattacacttgatggtgacacagtggtacctgtcgccccaacgctttctgcagaacagcttttggatgatggacttaagggattagcatgcatggatatctcatacggatgtgaggtggacgctagcaaccgatcagctggtgatcagagcatggattcttcacgatgcatcaatgagttatattgcgaggaaacggcagaagctatctgtgtactcaaaacatgtcttgtgctgaactgtatgcaattcaaacttgagatggatgatttagcacacaacgctactgagctggacaagatacagatgatgataccttttagtgaacgtgttttcagaatggcttcttcatttgctaccattgatgcccagtgtttcaggttttgtgtgatgatgaaggataagaatttgaagatagacatgcgtgaaacgatgagactttggactcgatcggcgttggacgattcagtggttacgtcatctttgagtatttcgctggatcgaggtcgatgggtagcagctgatgctactgatgctagattgctggtgtttccaattcgcgtgtaatgggtgagtgagccgatgtggtcgccaagacatgtgccggtgtcttggtggtgggtggcgcctaatcatc

SEQ ID NO: 10 - DNA, 1196 bp, Mammalian orthoreovirus
  source 1..1196: mol_type = other DNA
gctatttttgcctcttcccaaacgttgtcgcaatggaggtgtgcttgcccaacggtcatcagatcgtggacttgattaacaacgcttttgaaggtcgtgtatcaatctacagcgcgcaagagggatgggacaaaacaatctcagcacagccagatatgatggtatgtggtggtgccgtcgtttgcatgcattgtctaggtgttgttggatctctgcaacgcaagctgaagcatttgcctcaccatagatgtaatcaacagattcgtcatcaggattacgtcgatgtacagttcgcagatcgtgttactgctcactggaagcggggtatgctgtcctttgttgcgcagatgcacgcgatgatgaatgacgtatcaccagaggatctagaccgtgtgcgtactgagggaggttcactagtggagttaaactggcttcaggttgatccaaattcaatgtttagatcaatacactcaagttggacagatcctctgcaggtagtggatgatcttgacactaagctggatcaatactggacggccctgaatctgatgattgattcatccgacttggtgcccaacttcatgatgagagacccatcacatgcattcaatggtgtgagactggagggagacgcccgccaaactcaattctctaggactttcgattcgagatcgagtttagaatggggtgtgatggtttacgattactctgagttagagcatgatccatcgaagggccgtgcttacaggaaggaattggtgacgccagcacgagacttcggtcattttggattatcccactactctagggcgactaccccaatccttggaaagatgccagctgtattctcgggaatgttgactgggaattgtaaaatgtatccattcatcaaaggaacggctaagttaaagacagtgcgcaagctagtggattcagtcaatcatgcgtggggcgtcgagaagatcagatatgcgcttggaccaggtggcatgacgggatggtacgacaggactatgcagcaggcccccattgtactaactcccgctgctctcacaatgttctcagacaccaccaagttcggggatttggattatccggtgatgattggcgatccgatgattcttggctaaacacccccatcttcacagcgccgggcctgaccaacctggtgtgacgtgggacaggctccattcatc

SEQ ID NO: 11 - DNA, 3302 bp, Rotavirus
  source 1..3302: mol_type = other DNA
ggctattaaagctgtacaatggggaagtacaatctaatcttgtcagaatatctatcatttatatataattcacaatctgcagttcaaattccaatatattactcttccaacagtgaattagaaaatagatgtattgaatttcattccaagtgtttagagaactcaaagaatgggttatcgttaagaaagttgtttgttgaatataatgatgtcatagaaaatgccacattactgtcaatactatcatattcttacgacaagtataacgctgttgaaagaaaattggtgaagtatgcgaaaggcaaaccattggaggcagacttaacagtgaatgaattggattatgagaacaataaaataacatctgaattatttccaacagcggaggaatatacggactcactaatggatccagcaattttaacttcgctatcatcaaatttaaatgcagtcatgttctggttggaaaaacatgaaaatgatgtcgctgaaaaacttaaagtttataaaaggagattagacctattcaccatagtagcctcaacgataaataaatatggcgtaccaaggcataacgcaaagtacagatatgaatacgacgtaatgaaagataaaccgtactacttagtgacatgggcaaattcttcaattgaaatgttaatgtcagttttctctcatgacgactatttgatagcaaaagagttaatagtgttatcatattctaatagatctactctagcaaagttagtgtcatcaccaatgtcgattttggtagccttggtggatattaatggaacatttattacaaatgaagaattagaattggaattttcaaataaatatgtacgagcaatagttccggatcaaacatttgacgaattaaatcaaatgcttgacaatatgaggaaagctggattagttgacatacctaagatgatacaggactggttagttgatcgttctatcgaaaaatttccattaatggctaagatatattcatggtcgtttcatgttggatttagaaagcaaaaaatgctagatgctgcgctggatcaattgaaaactgagtatacagaaaatgtggacgatgaaatgtatcgggaatatacaatgttaataagagatgaagtagttaaaatgcttgaagaaccagttaaacatgatgatcacttgctacgagattctgagttagctggtttactatcaatgtcgtcagcatcgaatggtgagtcaaggcagctaaagtttggtaggaaaacaattttttcaactaaaaagaatatgcatgtcatggatgatatggctaacgaaagatacacgcctggtataataccaccagtgaatgttgataaaccaataccattaggaagaagagatgttccaggaagaaggactagaataatattcattctgccatacgaatatttcatagcacagcacgctgtagttgaaaaaatgttgatttacgcaaaacatacgagagaatacgctgaattttattcacaatcaaaccaattattgtcatacggcgatgtaacgcgttttttgtctaataacacaatggtcttgtatacggatgtatctcagtgggattcgtctcagcataatacacagccatttaggaaaggaataataatgggactggacatattagctaacatgactaatgatgctaaagttcttcagacattaaacttatacaaacaaacacaaatcaatctcatggattcatacgttcaaataccagatggcaacgtcattaagaaaatacaatacggggcagtagcatcaggagagaaacaaacgaaagcagcaaattcaatagcaaatttggcactgattaaaacggttttgtcacgtatttctaacaaacattcattcgcaacaaaaataataagagttgatggagatgataactatgcggtgctacaatttaatacagaggtgactaagcagatgatccaagacgtatcgaacgatgtaagagaaacttatgcacgcatgaatgctaaagttaaagctctggtatccacagtaggaatagaaattgctaaaaggtacattgcaggtggaaaaatattttttcgagctggaataaatctacttaataatgaaaagagagggcagagtacgcagtgggatcaagcagcaattttatattcaaattatattgtaaatagacttagaggatttgaaactgatagggagtttattttaactaagataatgcagatgacgtcagtcgcaattactggatcattaagactatttccttctgaacgcgtattaactacgaattcaacatttaaagtatttgactcggaggattttattatagagtacggaacgactgatgacgaagtatatatacaaagagcgttcatgtctttatcaagtcagaaatcaggaatagccgatgagatagcggcatcatcaacatttaaaaattacgtcacgagactatctgaacagttattattttcaaagaataatatagtgtccagaggaatagctttgactgaaaaagcgaaattgaattcatacgctccaatatcgcttgagaaaagacgtgcacagatatcagctttattgactatgttgcagaaaccggtcaccttcaaatcaagtaaaataacaataaatgacatactcagagatataaaaccattttttacagtaagtgatgcacacttacctatacaataccaaaaatttatgccaactttgccagataacgtacagtatataattcaatgtataggatccagaacttatcaaattgaagatgacggttcgaagtcagccatatctagactaatatcaaagtattcagtttataagccatcaattgaagaattgtataaagtgatttcattgcatgaaaacgaaatacaattatatctgatttcattaggaataccgaaaatagacgctgacacgtatgttggatcaaagatttattctcaagataagtatagaatactagaatcatacgtgtacaatttattgtccattaattatggatgctatcaattatttgatttcaattcaccggacttggagaagctgataagaataccatttaagggaaaaataccagctgttacattcatattacacttatatgcaaagctagaagttataaactacgctataaaaaatggttcatggataagcctattttgcaattaccctaaatcagaaatgataaaattatggaagaagatgtggaacatcacgtcattacgttcgccgtacactaacgcgaacttctttcaagattagaacgcttagatgtgacc

SEQ ID NO: 12 - DNA, 2693 bp, Rotavirus
  source 1..2693: mol_type = other DNA
ggctattaaaggctcaatggcgtatcgaaaacgtggagcgcgtcgtgagacgaatctaaaacaagatgaacgaatgcaagaaaaagaagatagcaagaacattaataatgacagtcctaaatcacaattatcagaaaaagtattatctaagaaagaagagataattacagataatcaagaagaagttaagatatctgatgaggtaaaaaaatctaataaagaagaatcgaaacagttgttagaagtacttaaaacaaaagaggaacatcaaaaagaagttcagtatgaaatattacaaaaaactatccctacatttgaaccaaaagagtcaatactcaaaaaattagaagacataaaaccagaacaagcaaagaaacaaactaaactgtttcgaatatttgaaccgaaacaattgcctatttatagagctaatggagaaagagagcttcgtaatagatggtattggaaattgaaacgagatactcttcctgatggagattatgatgttagagagtattttttaaatttatatgatcaagtattaatggaaatgccggattatctattacttaaagatatggctgtagagaataaaaattcaagggatgctggcaaagtagttgattctgaaacagccgcaatatgcgatgctatttttcaagatgaagaaaccgaaggtgcagtaagaagattcatagctgagatgagacaacgagttcaagctgatcgaaatgtagtcaattatccatctatattgcatccaattgaccatgcgtttaacgaatacttcttacaacatcagttggtagaaccattaaataatgatatcattttcaattacataccagagagaataagaaatgatgtcaactatatattaaatatggacaggaatttaccgtctactgctagatatatcagaccaaacttgctacaagataggttaaatttacatgataattttgagtcactctgggatactataactacatctaattatattttagcaagatctgtggtgccagacctaaaagaattagtatctactgaggcacaaatccagaaaatgtcacaagatttgcaattggaagctttgacaatacaatcagagactcagtttttaacaggtataaactcacaagccgctaatgattgttttaaaactttgattgctgctatgttgagtcagagaaccatgtcattagatttcgtaacgacaaattacatgtcacttatttcaggcatgtggttactcactgtgattccaaatgatatgtttataagagaatcattagtagcatgtcaactagccataataaataccattgtttatccggcattcggaatgcaaagaatgcattataggaatggtgatccacagactccctttcaaattgcagagcaacagattcaaaattttcaggtagctaattggttacattttgttaattataatcagtttagacaagtagtgattgatggagtgttaaatcaagtcttgaatgataatataagaaatggtcatgtagtcaaccaattaatggaagctctgatgcaattatctagacaacagtttcccacaatgccagttgattataaaagatctatacagagaggaattttgctgctttctaacagacttggtcagcttgtcgatttaacaagattgttatcatacaattatgagacattaatggcatgcataacaatgaatatgcagcatgttcaaacattaacaactgaaaaattgcaattaacatcagtaacatcattatgtatgctaattggaaatgctacggttataccgagtccgcaaacattgttccattactataatgtgaatgtcaattttcattcaaattataatgaaagaattaatgacgcagttgcaattataactgcggcaaatagattaaatttatatcaaaagaaaatgaaatcaatagttgaggactttctgaaaagattacagatatttgatgttgcgagagtaccagatgaccaaatgtatagattgagagatagattaagactattaccagttgaaataagaagattagatatttttaatttgatagcaatgaatatggaacagattgaacgtgcatcagataaaattgcacaaggagttataatagcataccgagatatgcagttagaacgagatgagatgtatggttacgtcaatattgccagaaacttggacggatttcaacaaataaatcttgaagaattgatgagatcaggagattatgctcaaattactaacatgctacttaataatcaaccagtagctttagttggagcgctaccatttataacggattcatcagtgatttcgttaatagctaaactagatgcaaccgtttttgcacagattgtcaaacttagaaaggtcgacacgttaaaacccatcctatataagataaattcagattctaatgacttttatttggtggctaattatgattggattcctacatctactacaaaagtgtataaacaagttccacaacaatttgattttagagcgtcaatgcatatgttaacgtctaacctaacatttaccgtatattcagatttgcttgcgttcgtttcagctgatactgttgaaccaattaatgctgttgcttttgataatatgcgcatcatgaacgaattgtaaacgccaaccccattgtggagatatgacc

SEQ ID NO: 13 - DNA, 2591 bp, Rotavirus
  source 1..2591: mol_type = other DNA
ggctattaaagcagtaccagtagtgtgttttacctctgatggtgtaaacatgaaagtactagctttaagacacagtgtggctcaagtgtatgcagacactcaagtctacgttcatgatgatacaaaagatagttatgaaaacgcttttttaatctctaatcttacgacccataatattttatacttaaattatagcattaaaacattagaaatattaaataagtcaggaatagctgcaattgctttacaatcacttgaagaattattcacattaataaggtgtaatttcacttatgattatgaacttgatataatatatttacatgattattcatattataccaataatgaaattagaacagaccaacattggataacaaaaacaaatattgaagaatatttactacctggatggaaattaacatatgttggttataatggaagtgaaactagaggacattataacttttcatttaaatgtcaaaacgctgcaacagatgatgatctaataattgaatacatttattcagaagcgttggacttccaaaattttatgttaaaaaagataaaggaaagaatgactacatcgttgcctatagctagattatctaacagagtatttagggataagttattcccatcattattgaaagaacataagaatgtagtgaacgttggtccgcgtaatgaatctatgtttacatttttaaattatccaactataaaacaattttcaaatggtgcgtatttagtaaaagatactataaaattaaaacaagaacgatggttaggtaaaaggatatctcagtttgatattggtcagtataaaaatatgctgaatgttcttacagcaatttattattactataatttatataaaagtaaaccaattatatatatgatcggatctgctccatcttattggatatatgacgttaggcattattccgattttttctttgaaacttgggatccattggacacaccatattcatcaatccatcacaaagaattattttttataaatgatgtgaagaaactgaaggataactcaatattgtatattgatataagaaccgataggggcaatgctgattggaaaaaatggagaaagacagtagaagaacaaactattaataatttggacatagcttatgaatatttacgaacgggtaaagcgaaggtgtgttgtgttaagatgacagctatggatttggaactgccaatttcagctaaattactgcaccacccaactacggaaataagatcagaattttatttattactagatacttgggatttaactaacattaggaggttcattcctaaaggcgtgttatattcatttataaacaatataataactgaaaatgtgtttattcaacaaccatttaaagtaaaagtactgaatgatagttatattgtagcgttatatgcattatcaaatgattttaataatagatcagaagtaattaaattaattaataatcagaaacaatctctaataactgttagaataaataatacgtttaaggatgaaccaaaagttgggttcaaaaatatctatgattggacctttcttccaaccgactttgataccaaagaagctataattacttcatacgacggttgtttaggactctttggtttgtctatatcgttagcatcaaaaccaacagggaataatcatttattcattttaagtggtacagataagtattataaattggatcaatttgctaatcacaccagtatatcgagaagatcacaccaaattaggttttcggaatctgctacttcatattcaggttatatatttagagatttgtccaataataattttaatctaattggtactaatatagagaattcagtatcaggtcatgtatataatgctttaatttattatagatataattattcatttgatcttaaacgctggatttatttacattctatagataaagttgatatagaaggaggaaagtattatgaacacgcaccaatagaattaatttatgcatgtagatcagcaaaagaatttgctacattgcaggatgacttaactgtattgagatattcaaacgaaatagagaattatattaatacagtatatagtataacatacgctgatgatccgaattactttatcggaatacaatttagaaatataccatataaatatgatgttaaaataccgcatttaaccttcggagtattacatatttctgataacatggtgccagacgtgattgacatactaaagataatgaagaatgaattatttaaaatggatattacgaccagttatacatatatgttatcagatggaatctacgtagcaaatgttagtggagtattatctacatactttaaaatctataacgtattttataaaaatcaaataacttttggccaatccagaatgtttattccgcacataacattaagcttcaataacatgagaacagtaaggatagagactactaaattacaaattaaatccatttatttaagaaagattaagggtgatacagtgtttgatatggttgagtgagctaaaaacttaacacactagtcatgatgtgacc

SEQ ID NO: 14 - DNA, 2362 bp, Rotavirus
  source 1..2362: mol_type = other DNA
ggctataaaatggcttcgctcatttatagacaattgctcacgaattcttatacagtagatttatccgatgagatacaagagattggatcaactaaatcacaaaatgtcacaattaatcctggaccatttgcgcaaacaggttatgctccagttaactggggacctggagaaattaatgattctacgacagttggaccattgctggatgggccttatcaaccaacgacattcaatccaccagtcgattattggatgttactggctccaacgacacctggcgtaattgttgaaggtacaaataatacagatagatggttagccacaattttaatcgagccaaatgttcagtctgaaaatagaacttacactatatttggtattcaagaacaattaacggtatccaatacttcacaagaccagtggaaatttattgatgtcgtaaaaacaactgcaaatggaagtataggacaatatggaccattactatccagtccgaaattatatgcagttatgaagcataatgaaaaattatatacatatgaaggacagacacctaacgctaggacagcacattattcaacaacgaattatgattctgttaacatgactgctttttgtgacttttatataattcctagatctgaagagtctaaatgtacggaatacattaataatggattaccaccaatacaaaatactagaaatgttgtaccattatcgttgactgctagagatgtaatacactatagagctcaagctaatgaagatattgtgatatccaagacatcattatggaaagaaatgcaatataatagagatataactattagatttaaatttgcaaatacaattataaaatcaggagggctgggatataagtggtcagaaatatcatttaagccagcgaattatcaatacacatatactcgtgatggtgaagaagttaccgcacatactacttgttcagtgaatggcgttaatgacttcagttttaatggaggatatttaccaactgattttgttgtatctaaatttgaagtaattaaagagaattcatacgtctatatcgattactgggatgattcacaagcatttcgtaacgtggtgtatgtccgatcgttagcagcaaacttgaattcagttatgtgtactggaggcagctataattttagtctaccagttggacaatggcctgttttaactgggggagcagtttctttacattcagctggtgtaacactatctactcaatttacagatttcgtatcattaaattcattaagatttagatttagactagctgtcgaagaaccacactttaaactgactagaactagattagatagattgtatggtctgcctgctgcagatccaaataatggtaaagaatattatgaaattgctggacgattttcacttatatcattagtgccatcaaatgatgactatcagactcctatagcaaactcagttactgtacgacaagatttagaaaggcagttaggagaactaagagaagagtttaacgctttgtctcaagaaattgcaatgtcgcagttaatcgatttagcgcttctaccattagatatgttctcaatgttttctggcattaaaagtactattgatgctgcaaaatcaatggctactaatgttatgaaaaaattcaaaaagtcaggattagcgaattcagtttcaacactgacagattctttatcagacgcagcatcatcaatatcaagaggttcatctatacgttcgattggatcttcagcatcagcatggacggatgtatcaacacaaataactgatatatcgtcatcagtaagttcagtttcgacacaaacgtcaactatcagtagaagattgagactaaaggaaatggcaacacaaactgagggtatgaattttgatgatatatcagcggctgttttgaagactaagatagataaatcgactcaaatatcaccaaacacaatacctgacattgttactgaagcatcggaaaaattcataccaaatagggcttaccgcgttataaacaacgatgatgtgtttgaagctggaattgatgggaaattttttgcttataaagtggatacatttgaggaaataccatttgatgtacaaaaattcgctgacttagttacagattctccagtaatatccgctataattgattttaaaacacttaaaaatttgaacgataattacggcattactaagcaacaagcatttaatcttttaagatctgacccaagagttttacgtgaattcattaatcaggacaatcctataattagaaatagaattgaacaactgattatgcaatgcaggttgtgagtaatttctagaggatgtgacc

SEQ ID NO: 15 - DNA, 1610 bp, Rotavirus
  source 1..1610: mol_type = other DNA
ggcttttttttgaaaagtcttgtgttagccatggctacttttaaagatgcatgctttcattatcgtagattaactgctttaaatcggagattatgcaacattggtgcaaattctatttggatgccagttcctgatgcgaaaattaaggggtggtgtttagaatgttgtcaaatagctgatttaacccattgttatggttgctcattgccgcatgtttgcaaatggtgtgttcagaacagaagatgcttccttgacaatgaacctcatttgcttaagcttagaactgtgaaacatccaattaccaaagacaaattacagtgtatcatagacttgtacaatataatatttccaattaatgataaagtaattagaaaatttgaaagaatgataaagcaaagagaatgtaggaatcaatataaaattgaatggtataatcatttgctgctcccaattacattaaatgctgctgcatttaagtttgatgaaaataatctttattatgtttttgggttatatgagaaatcagtcagtgatatatatgctccatatagaattgttaactttataaatgaatttgataaattattgcttgatcatattaactttacaagaatgtccaatctaccaatagagttgagaaaccattacgcaaagaaatacttccaattatcaagactgccatcatcaaaactaaagcaaatttacttttcagattttactaaagaaactgtgatttttaatacttatacaaaaacgccaggaagatcaatatacagaaatgtaactgaatttaattggagagatgaattggagctttattctgatttaaaaaatgataagaataaattaattgctgcaatgatgacgagtaagtatactcggttctatgctcatgataataattttggaaggttgaaaatgacaatatttgagttgggacatcattgtcagcctaactacgtggcatctaatcacccaggcaatgcttccgatatccagtactgtaaatggtgtaatataaaatattttcttagtaaaattgattggcggattcgtgatatgtataatttattgatggaatttattaaggattgttataaaagtaatgttaacgttggacattgtagttctgttgaaaacatatatcctttaattaaaagattaatttggagtttgtttactaatcacatggatcaaacaattgaagaagtgtttaatcacatgtcgccagtgtcagttgaaggtacgaatgtcatcatgttgattcttggattgaatattagtttgtataatgaaattaagcgcactttgaatgtagatagcataccaatggtacttaatttaaatgaattcagtagtatagttaaatcaattagcagtaaatggtataatgttgatgaattggataaattgccaatgtcaataaaatcaacggaggaactgattgaaatgaagaattctggaactttaactgaagaatttgagctactgatctccaactcagaagatgacaatgagtgaaattatgtcactatctaattatacagtatttagccatcacaagaccgtccagactagagtagcgcctagctggcaaaatactgtgaacc

SEQ ID NO: 16 - DNA, 1356 bp, Rotavirus
  source 1..1356: mol_type = other DNA
ggcttttaaacgaagtcttcaacatggatgtcctatactctttgtcaaagactcttaaagacgctagagacaaaattgtcgaaggcacattgtattctaacgtgagtgatctaattcaacaatttaatcaaatgataattactatgaatggaaatgaatttcaaactggaggaatcggtaatttgccaattagaaactggaattttaatttcgggttacttggaacaactttgctgaacttagacgctaattatgttgaaacggcaagaaatacaattgattatttcgtggattttgtagacaatgtatgcatggatgagatggttagagaatcacaaaggaacggaattgcacctcaatcagactcgctaagaaagctgtcagccattaaattcaaaagaataaattttgataattcgtcggaatacatagaaaactggaatttgcaaaatagaagacagaggacaggtttcacttttcataaaccaaacatttttccttattcagcatcatttacactaaatagatcacaacccgctcatgataatttgatgggcacaatgtggttaaacgcaggatcggaaattcaagtcgctggatttgactactcatgtgctattaacgcaccagccaatatacaacaatttgagcatattgtgccactccgaagagtgttaactacagctacgataactcttctaccagacgcggaaaggtttagttttccaagagtgatcaattcagctgacggggcaactacatggtttttcaacccagtgattctcaggccgaataacgttgaagtggagtttctattgaatggacagataataaacacttatcaagcaagatttggaactatcgtagctagaaattttgatactattagactatcattccagttaatgagaccaccaaacatgacaccagcagtagcagtactattcccgaatgcacagccattcgaacatcatgcaacagtgggattgacacttagaattgagtctgcagtttgtgagtctgtactcgccgatgcaagtgaaactctattagcaaatgtaacatccgttaggcaagagtacgcaataccagttggaccagtctttccaccaggtatgaactggactgatttaatcaccaattattcaccgtctagggaggacaatttgcaacgcgtatttacagtggcttccattagaagcatgctcattaaatgaggaccaagctaacaacttggtatccaactttggtgagtatgtagctatatcaagctgtttgaactctgtaagtaaggatgcgtatacgcattcgctacacagagtaatcactcagatggtatagtgagaggatgtgacc

SEQ ID NO: 17 - DNA, 1105 bp, Rotavirus
  source 1..1105: mol_type = other DNA
ggcatttaatgcttttcagtggttgatgctcaagatggagtctacgcaacagatggccgtctcaattattaactcttcttttgaagctgcagttgtagctgcaacctcagctcttgagaatatgggaatagaatatgattatcaggatatatattctagagtaaagaataaatttgattttgtgatggacgattctggtgttaaaaataatctgattggtaaagcaataactattgatcaagctttgaataataaatttggatctgctataagaaatagaaactggcttgctgatacttctagagcagctaaattagatgaggatgtaaacaaactaagaatgatgttatcatcaaaaggaattgatcaaaaaatgagagttttaaacgcatgcttcagtgtaaaaagaatacctggaaaatcatcatctattattaaatgcacaaaattgatgcgtgataaattggaacgtggtgaagttgaagtggatgattcatttgtggatgaaaaaatggaagtggataccattgactggaaatcgcgctatgagcaattggagcaaaggtttgaatcattgaaatccagggtaaatgaaaaatataataattgggtgttgaaagcaagaaaaatgaatgaaaatatgcattctcttcaaaatgtcatctctcaacagcaagcacatatagctgagcttcaagtgtacaataataaactagaacgtgatttgcaaaataaaattggatcccttacttcttcgattgaatggtatttaagatcaatggaattagaccctgaaataaaggcagacattgaacagcaaattaactcaattgatgcgataaatccattgcacgcttttgatgacttagaatcagtaatacgtaatttgatatctgattatgacaaattattccttatgttcaaaggattaatacagagatgtaattatcaatattcatttggttgcgaataaccattttgatacatgttgaacaatcaaatacagtgttagtatgttgtcatctatgcataaccctctatgagcacaatagttaaaagctaacactgtcaaaaacctaaatggctataggggcgttatgtggcc

SEQ ID NO: 18 - DNA, 1059 bp, Rotavirus
  source 1..1059: mol_type = other DNA
ggcttttaaagcgtctcagtcgccgtttgagccttgcggtgtagccatggctgagctagcttgcttttgctatcctcatttggagaatgatagctataaatttattccttttaataatttagctattaaagctatgctgacagctaaagtagacaaaaaggacatggataagttttatgattcaattatttatggaatagcaccgcctcctcaatttaagaaacggtataatactaatgataattcaagaggcatgaattttgaaacaattatgtttactaaggtggctatgttgatatgtgaagctctaaattcattgaaagtgacgcaagcaaacgtctctaatgtattatcacgagtagtatcaataaggcatttagaaaatttggtgatacgtaaagaaaatccacaggatattctatttcattcaaaagatttacttttgaaatcaacactgattgctattggacagtctaaagaaattgaaactacaataactgcagaaggaggagaaattgtatttcaaaacgctgccttcaccatgtggaaactaacttatttagaacatcaattgatgccaattctggatcagaattttattgaatataaagttacattgaacgaagataaaccaatttcagatgttcatgttaaagaattagtcgctgaacttcgatggcaatataacaagtttgctgtaatcacacatggtaagggtcattatagaattgtaaagtattcatcagttgctaatcacgctgacagagtatatgcaactttcaagagtaatgttaaaactggagttaataatgattttaacctacttgatcaaagaattatttggcaaaactggtatgcatttacatcatcaatgaaacagggtaatacacttgacgtgtgtaaaaggttgcttttccaaaaaatgaaaccagaaaaaaatccatttaaagggctgtcaacggatagaaaaatggacgaagtttctcaagttggcgtttaattcgctatcaatttgaggatgatgatggcttagcaagaatagaaagcgcttatgtgacc

SEQ ID NO: 19 - DNA, 1063 bp, Rotavirus
  source 1..1063: mol_type = other DNA
ggctttaaaaagagagaatttccgtttggctagcggttagctccttttaatgtatggtattgaatataccacagttctaacctttctgatatcgattattctactaaattacatacttaaatcattaactagaataatggactttataatttatagatttctttttataattgtgatattgtcaccatttctcagagcacaaaattatggtattaatcttccaatcacaggctccatggacattgcatacgctaattcaacgcaagaagaaccattcctcacttctacactttgcctatattatccgactgaggctgcgactgaaataaacgataattcatggaaagacacactgtcacaactatttcttacgaaagggtggccaactggatccgtatattttaaagaatatactaacattgcatcgttttctgttgatccgcagttgtattgtgattataacgtagtactaatgaaatatgacgcgacgttgcaattggatatgtcagaacttgcggatctaatattaaacgaatggttgtgtaatccaatggatattactctgtattattatcagcaaactgacgaagcgaataaatggatatcaatgggctcatcatgtacaattaaagtatgtccacttaatacacaaactcttggaattggatgcttgacaactgatgctacaacttttgaagaagttgcgacagctgaaaagttggtaattactgacgtggttgatggcgttaatcataagctggatgtcacaacagcaacgtgtactattagaaactgtaagaaattgggaccaagagaaaacgtagccgttatacaagttggtggttctgacatcctcgatataactgctgatccaactactgcaccacagacagaacggatgatgcgaattaactggaaaaaatggtggcaagttttttatactgtagtagactatgtagatcagataatacaagttatgtccaaaagatcaagatcactaaattcagcagcattttattacagagtgtaggtataacttaggttagaattgtatgatgtgacc

SEQ ID NO: 20 - DNA, 751 bp, Rotavirus
  source 1..751: mol_type = other DNA
ggcttttaaaagttctgttccgagagagcgcgtgcggaaagatggaaaagcttaccgacctcaattatacattgagtgtaatcactctaatgaacaatacattgcacacaatacttgaggatccaggaatggcgtattttccttatatagcatctgtcttaacagttttgtttgcgctacataaagcatccattccaacaatgaaaattgcattgaaaacgtcaaaatgttcatataaagtggtgaaatattgtattgtaacaatttttaatacgttgttaaaattggcaggttataaagagcagataactactaaagatgagatagaaaagcaaatggacagagtagtcaaagaaatgagacgccagctagaaatgattgacaaattgactacacgtgaaattgaacaagtagagttgcttaaacgcatttacgataaattgacggtgcaaacgacaggtgaaatagatatgacaaaagagatcaatcaaaaaaacgtgagaacgctagaagaatgggaaagtggaaaaaatccttatgaaccaagagaagtgactgcagcaatgtaagaggttgagctgccgtcgactgtcctcggaagcggcggagttctttacagtaagcaccatcggacctgatggctgactgagaagccacagtcagccatatcgcgtgtggctcaagccttaatcccgtttaaccaatccggtcagcaccggacgttaatggaaggaacggtcttaatgtgacc

SEQ ID NO: 21 - DNA, 667 bp, Rotavirus
  source 1..667: mol_type = other DNA
ggcttttaaagcgctacagtgatgtctctcagtattgacgtgacgagtcttccttctattccttcaactatatataagaatgaatcgtcttcaacaacgtcaactctttctggaaaatctattggtaggagtgaacagtacatttcaccagatgcagaagcattcaataaatacatgctgtcgaagtctccagaggatattggaccatctgattctgcttcaaacgatccactcaccagtttttcgattagatcgaatgcagttaagacaaacgcagacgctggcgtgtctatggattcatcagcacaatcacgaccttcaagtaatgtcggatgcgatcaagtggatttctccttaaataaaggcttaaaagtaaaagctaatttggactcatcaatatcaatatctacggatactaaaaaggagaaatcaaaacaaaaccataaaagtaggaagcactacccaagaattgaagcagagtctgattcagatgattatgtactggatgattcagatagtgatgatggtaaatgtaagaactgtaaatataagaagaaatacttcgcattaagaatgagaatgaaacaagtcgcaatgcaattgattgaagatttgtaagtctgacctgggaacacactagggagctccccactcccgttttgtgacc

SEQ ID NO: 22 - DNA, 17 bp, T7 phage
  source 1..17: mol_type = other DNA
taatacgactcactata

SEQ ID NO: 23 - DNA, 83 bp, Hepatitis D virus
  source 1..83: mol_type = other DNA
gggtcggcatggcatctccacctcctcgcggtccgacctgggcatccgaaggaggacgtcgtccactcggatggctaagggag

SEQ ID NO: 24 - DNA, 151 bp, T7 phage
  source 1..151: mol_type = other DNA
agctcaaaaaaaaggatccggctgctaacaaagcccgaaaggaagctgagttggctgctgccaccgctgagcaataactagcataaccccttggggcctctaaacgggtcttgaggggttttttgctgaaaggaggaactatatccggatc

SEQ ID NO: 25 - DNA, 3076 bp, synthetic construct
  misc_feature 1..3076: note = p3E5 plasmid
  source 1..3076: mol_type = other DNA
atcgatcccgggttaatacgactcactatagggtcggcatggcatctccacctcctcgcggtccgacctgggcatccgaaggaggacgtcgtccactcggatggctaagggagagctcaaaaaaaaggatccggctgctaacaaagcccgaaaggaagctgagttggctgctgccaccgctgagcaataactagcataaccccttggggcctctaaacgggtcttgaggggttttttgctgaaaggaggaactatatccggatcgagatcctctagagtcgacctgcaggcatgcaagcttgtattctatagtgtcacctaaatcgtatgtgtatgatacataaggttatgtattaattgtagccgcgttctaacgacaatatgtacaagcctaattgtgtagcatctggcttactgaagcagaccctatcatctctctcgtaaactgccgtcagagtcggtttggttggacgaaccttctgagtttctggtaacgccgttccgcaccccggaaatggtcagcgaaccaatcagcagggtcatcgctagccagatcctctacgccggacgcatcgtggccggcatcaccggcgccacaggtgcggttgctggcgcctatatcgccgacatcaccgatggggaagatcgggctcgccacttcgggctcatgagcgcttgtttcggcgtgggtatggtggcaggccccgtggccgggggactgttgggcgccatctccttgcaccattccttgcggcggcggtgctcaacggcctcaacctactactgggctgcttcctaatgcaggagtcgcataagggagagcgtcgatatggtgcactctcagtacaatctgctctgatgccgcatagttaagccagccccgacacccgccaacacccgctgacgcgccctgacgggcttgtctgctcccggcatccgcttacagacaagctgtgaccgtctccgggagctgcatgtgtcagaggttttcaccgtcatcaccgaaacgcgcgagacgaaagggcctcgtgatacgcctatttttataggttaatgtcatgataataatggtttcttagacgtcaggtggcacttttcggggaaatgtgcgcggaacccctatttgtttatttttctaaatacattcaaatatgtatccgctcatgagacaataaccctgataaatgcttcaataatattgaaaaaggaagagtatgagtattcaacatttccgtgtcgcccttattcccttttttgcggcattttgccttcctgtttttgctcacccagaaacgctggtgaaagtaaaagatgctgaagatcagttgggtgcacgagtgggttacatcgaactggatctcaacagcggtaagatccttgagagttttcgccccgaagaacgttttccaatgatgagcacttttaaagttctgctatgtggcgcggtattatcccgtattgacgccgggcaagagcaactcggtcgccgcatacactattctcagaatgacttggttgagtactcaccagtcacagaaaagcatcttacggatggcatgacagtaagagaattatgcagtgctgccataaccatgagtgataacactgcggccaacttacttctgacaacgatcggaggaccgaaggagctaaccgcttttttgcacaacatgggggatcatgtaactcgccttgatcgttgggaaccggagctgaatgaagccataccaaacgacgagcgtgacaccacgatgcctgtagcaatggcaacaacgttgcgcaaactattaactggcgaactacttactctagcttcccggcaacaattaatagactggatggaggcggataaagttgcaggaccacttctgcgctcggcccttccggctggctggtttattgctgataaatctggagccggtgagcgtgggtctcgcggtatcattgcagcactggggccagatggtaagccctcccgtatcgtagttatctacacgacggggagtcaggcaactatggatgaacgaaatagacagatcgctgagataggtgcctcactgattaagcattggtaactgtcagaccaagtttactcatatatactttagattgatttaaaacttcatttttaatttaaaaggatctaggtgaagatcctttttgataatctcatgaccaaaatcccttaacgtgagttttcgttccactgagcgtcagaccccgtagaaaagatcaaaggatcttcttgagatcctttttttctgcgcgtaatctgctgcttgcaaacaaaaaaaccaccgctaccagcggtggtttgtttgccggatcaagagctaccaactctttttccgaaggtaactggcttcagcagagcgcagataccaaatactgtccttctagtgtagccgtagttaggccaccacttcaagaactctgtagcaccgcctacatacctcgctctgctaatcctgttaccagtggctgctgccagtggcgataagtcgtgtcttaccgggttggactcaagacgatagttaccggataaggcgcagcggtcgggctgaacggggggttcgtgcacacagcccagcttggagcgaacgacctacaccgaactgagatacctacagcgtgagctatgagaaagcgccacgcttcccgaagggagaaaggcggacaggtatccggtaagcggcagggtcggaacaggagagcgcacgagggagcttccagggggaaacgcctggtatctttatagtcctgtcgggtttcgccacctctgacttgagcgtcgatttttgtgatgctcgtcaggggggcggagcctatggaaaaacgccagcaacgcggcctttttacggttcctggccttttgctggccttttgctcacatgttctttcctgcgttatcccctgattctgtggataaccgtattaccgcctttgagtgagctgataccgctcgccgcagccgaacgaccgagcgcagcgagtcagtgagcgaggaagcggaagagcgcccaatacgcaaaccgcctctccccgcgcgttggccgattcattaatgcagggggat

SEQ ID NO: 26 - DNA, 288 bp, Nelson bay reovirus
  source 1..288: mol_type = other DNA
atgagcggtgattgcgctggtctggtttcagtgtttgggagtgttcactgtcagtcgtctaagaataaagccggtggggatctgcaagcgacttctgttctaaccacatattggccgcatcttgcgattggtggcagtatcatcttgatcatcctcctgctgggtctattttactgttgttatctcaagtggaagacgtcacatattcgtcgtacttatcacaaggagttggtggcgctaactcgcggctatgtcaggccgatcccggcggacgttaccagtgtctga

SEQ ID NO: 27 - DNA, 297 bp, Avian reovirus
  source 1..297: mol_type = other DNA
atgctgcgtatgcctcccggttcgtgtaacggtgcgactgctgtatttggtaacgttcattgtcaggcagctcaaaacacggcaggtggtgatttgcaagctacgtcatccataattgcatattggccttatctagcggcgggtggtggtttcttattaattgttatcattttcgctcttctatactgttgtaaggctaaggtcaaggcggacgctgcacgtagtgtcttccatcgtgagctggtagcgttgagttctggtaagcacaatgcaatggctccgccatacgacgtttga

SEQ ID NO: 28 - DNA, 5699 bp, synthetic construct
  misc_feature 1..5699: note = pCAGPM plasmid
  source 1..5699: mol_type = other DNA
gtcgacattgattattgactagttattaatagtaatcaattacggggtcattagttcatagcccatatatggagttccgcgttacataacttacggtaaatggcccgcctggctgaccgcccaacgacccccgcccattgacgtcaataatgacgtatgttcccatagtaacgccaatagggactttccattgacgtcaatgggtggactatttacggtaaactgcccacttggcagtacatcaagtgtatcatatgccaagtacgccccctattgacgtcaatgacggtaaatggcccgcctggcattatgcccagtacatgaccttatgggactttcctacttggcagtacatctacgtattagtcatcgctattaccatgggtcgaggtgagccccacgttctgcttcactctccccatctcccccccctccccacccccaattttgtatttatttattttttaattattttgtgcagcgatgggggcggggggggggggggcgcgcgccaggcggggcggggcggggcgaggggcggggcggggcgaggcggagaggtgcggcggcagccaatcagagcggcgcgctccgaaagtttccttttatggcgaggcggcggcggcggcggccctataaaaagcgaagcgcgcggcgggcgggagtcgctgcgttgccttcgccccgtgccccgctccgcgccgcctcgcgccgcccgccccggctctgactgaccgcgttactcccacaggtgagcgggcgggacggcccttctcctccgggctgtaattagcgcttggtttaatgacggctcgtttcttttctgtggctgcgtgaaagccttaaagggctccgggagggccctttgtgcgggggggagcggctcggggggtgcgtgcgtgtgtgtgtgcgtggggagcgccgcgtgcggcccgcgctgcccggcggctgtgagcgctgcgggcgcggcgcggggctttgtgcgctccgcgtgtgcgcgaggggagcgcggccgggggcggtgccccgcggtgcgggggggctgcgaggggaacaaaggctgcgtgcggggtgtgtgcgtgggggggtgagcagggggtgtgggcgcggcggtcgggctgtaacccccccctgcacccccctccccgagttgctgagcacggcccggcttcgggtgcggggctccgtgcggggcgtggcgcggggctcgccgtgccgggcggggggtggcggcaggtgggggtgccgggcggggcggggccgcctcgggccggggagggctcgggggaggggcgcggcggccccggagcgccggcggctgtcgaggcgcggcgagccgcagccattgccttttatggtaatcgtgcgagagggcgcagggacttcctttgtcccaaatctggcggagccgaaatctgggaggcgccgccgcaccccctctagcgggcgcgggcgaagcggtgcggcgccggcaggaaggaaatgggcggggagggccttcgtgcgtcgccgcgccgccgtccccttctccatctccagcctcggggctgccgcagggggacggctgccttcgggggggacggggcagggcggggttcggcttctggcgtgtgaccggcggctctagagcctctgctaaccatgttcatgccttcttctttttcctacagctcctgggcaacgtgctggttgttgtgctgtctcatcattttggcaaagaattcgaagatcttaagatatcggcgcgccgtttaaacttaattaattcactcctcaggtgcaggctgcctatcagaaggtggtggctggtgtggccaatgccctggctcacaaataccactgagatcgatctttttccctctgccaaaaattatggggacatcatgaagccccttgagcatctgacttctggctaataaaggaaatttattttcattgcaatagtgtgttggaattttttgtgtctctcactcggaaggacatatgggagggcaaatcatttaaaacatcagaatgagtatttggtttagagtttggcaacatatgccatatgctggctgccatgaacaaaggtggctataaagaggtcatcagtatatgaaacagccccctgctgtccattccttattccatagaaaagccttgacttgaggttagattttttttatattttgttttgtgttatttttttctttaacatccctaaaattttccttacatgttttactagccagatttttcctcctctcctgactactcccagtcatagctgtccctcttctcttatgaagatccctcgacctgcagcccaagctctgtggaatgtgtgtcagttagggtgtggaaagtccccaggctccccagcaggcagaagtatgcaaagcatgcatctcaattagtcagcaaccaggtgtggaaagtccccaggctccccagcaggcagaagtatgcaaagcatgcatctcaattagtcagcaaccatagtcccgcccctaactccgcccatcccgcccctaactccgcccagttccgcccattctccgccccatggctgactaattttttttatttatgcagaggccgaggccgcctcggcctctgagctattccagaagtagtgaggaggcttttttggaggcctaggcttttgcaaaaagcttgcatgcctgcaggtcggccgccacgaccggtgccgccaccatcccctgacccacgcccctgacccctcacaaggagacgaccttccatgaccgagtacaagcccacggtgcgcctcgccacccgcgacgacgtcccccgggccgtacgcaccctcgccgccgcgttcgccgactaccccgccacgcgccacaccgtcgacccggaccgccacatcgagcgggtcaccgagctgcaagaactcttcctcacgcgcgtcgggctcgacatcggcaaggtgtgggtcgcggacgacggcgccgcggtggcggtctggaccacgccggagagcgtcgaagcgggggcggtgttcgccgagatcggcccgcgcatggccgagttgagcggttcccggctggccgcgcagcaacagatggaaggcctcctggcgccgcaccggcccaaggagcccgcgtggttcctggccaccgtcggcgtctcgcccgaccaccagggcaagggtctgggcagcgccgtcgtgctccccggagtggaggcggccgagcgcgccggggtgcccgccttcctggagacctccgcgccccgcaacctccccttctacgagcggctcggcttcaccgtcaccgccgacgtcgaggtgcccgaaggaccgcgcacctggtgcatgacccgcaagcccggtgcctgacgcccgccccacgacccgcagcgcccgaccgaaaggagcgcacgaccccatggctccgaccgaagccgacccgggcggccccgccgaccccgcacccgcccccgaggcccaccgactctagaggatcataatcagccataccacatttgtagaggttttacttgctttaaaaaacctcccacacctccccctgaacctgaaacataaaatgaatgcaattgttgttgttaacttgtttattgcagcttataatggttacaaataaagcaatagcatcacaaatttcacaaataaagcatttttttcactgcattctagttgtggtttgtccaaactcatcaatgtatcttatcatgtctggatccgctgcattaatgaatcggccaacgcgcggggagaggcggtttgcgtattgggcgctcttccgcttcctcgctcactgactcgctgcgctcggtcgttcggctgcggcgagcggtatcagctcactcaaaggcggtaatacggttatccacagaatcaggggataacgcaggaaagaacatgtgagcaaaaggccagcaaaaggccaggaaccgtaaaaaggccgcgttgctggcgtttttccataggctccgcccccctgacgagcatcacaaaaatcgacgctcaagtcagaggtggcgaaacccgacaggactataaagataccaggcgtttccccctggaagctccctcgtgcgctctcctgttccgaccctgccgcttaccggatacctgtccgcctttctcccttcgggaagcgtggcgctttctcaatgctcacgctgtaggtatctcagttcggtgtaggtcgttcgctccaagctgggctgtgtgcacgaaccccccgttcagcccgaccgctgcgccttatccggtaactatcgtcttgagtccaacccggtaagacacgacttatcgccactggcagcagccactggtaacaggattagcagagcgaggtatgtaggcggtgctacagagttcttgaagtggtggcctaactacggctacactagaaggacagtatttggtatctgcgctctgctgaagccagttaccttcggaaaaagagttggtagctcttgatccggcaaacaaaccaccgctggtagcggtggtttttttgtttgcaagcagcagattacgcgcagaaaaaaaggatctcaagaagatcctttgatcttttctacggggtctgacgctcagtggaacgaaaactcacgttaagggattttggtcatgagattatcaaaaaggatcttcacctagatccttttaaattaaaaatgaagttttaaatcaatctaaagtatatatgagtaaacttggtctgacagttaccaatgcttaatcagtgaggcacctatctcagcgatctgtctatttcgttcatccatagttgcctgactccccgtcgtgtagataactacgatacgggagggcttaccatctggccccagtgctgcaatgataccgcgagacccacgctcaccggctccagatttatcagcaataaaccagccagccggaagggccgagcgcagaagtggtcctgcaactttatccgcctccatccagtctattaattgttgccgggaagctagagtaagtagttcgccagttaatagtttgcgcaacgttgttgccattgctacaggcatcgtggtgtcacgctcgtcgtttggtatggcttcattcagctccggttcccaacgatcaaggcgagttacatgatcccccatgttgtgcaaaaaagcggttagctccttcggtcctccgatcgttgtcagaagtaagttggccgcagtgttatcactcatggttatggcagcactgcataattctcttactgtcatgccatccgtaagatgcttttctgtgactggtgagtactcaaccaagtcattctgagaatagtgtatgcggcgaccgagttgctcttgcccggcgtcaatacgggataataccgcgccacatagcagaactttaaaagtgctcatcattggaaaacgttcttcggggcgaaaactctcaaggatcttaccgctgttgagatccagttcgatgtaacccactcgtgcacccaactgatcttcagcatcttttactttcaccagcgtttctgggtgagcaaaaacaggaaggcaaaatgccgcaaaaaagggaataagggcgacacggaaatgttgaatactcatactcttcctttttcaatattattgaagcatttatcagggttattgtctcatgagcggatacatatttgaatgtatttagaaaaataaacaaataggggttccgcgcacatttccccgaaaagtgccacctg

SEQ ID NO: 29 - DNA, 2535 bp, Vaccinia virus
  source 1..2535: mol_type = other DNA
atggatgccaacgtagtatcatcttctactattgcgacgtatatagacgctttagcgaagaatgcttcggaattagaacagaggtctaccgcatacgaaataaataatgaattggaactagtatttattaagccgccattgattactttgacaaatgtagtgaatatctctacgattcaggaatcgtttattcgatttaccgttactaataaggaaggtgttaaaattagaactaagattccattatctaaggtacatggtctagatgtaaaaaatgtacagttagtagatgctatagataacatagtttgggaaaagaaatcattagtgacggaaaatcgtcttcacaaagaatgcttgttgagactatcgacagaggaacgtcatatatttttggattacaagaaatatggatcctctatccgactagaattagtcaatcttattcaagcaaaaacaaaaaactttacgatagactttaagctaaaatattttctaggatccggtgcccagtctaaaagttctttattacacgctattaatcatccaaagtcaaggcctaatacatctctggaaatagaatttacacctagagacaatgaaacagttccatatgatgaactaataaaggaattgacgactctctcgcgtcatatatttatggcttctccagagaatgtaattctttctccgcctattaacgcgcctataaaaacctttatgttgcctaaacaagatatagtaggtttggatctggaaaatctatatgccgtaactaagactgacggcattcctataactatcagagttacatcaaacgggttgtattgttattttacacatcttggttatattattagatatcctgttaagagaataatagattccgaagtagtagtctttggtgaggcagttaaggataagaactggaccgtatatctcattaagctaatagagcctgtgaatgcaatcaatgatagactagaagaaagtaagtatgttgaatctaaactagtggatatttgtgatcggatagtattcaagtcaaagaaatacgaaggtccgtttactacaactagtgaagtcgtcgatatgttatctacatatttaccaaagcaaccagaaggtgttattctgttctattcaaagggacctaaatctaacattgattttaaaattaaaaaggaaaatactatagaccaaactgcaaatgtagtatttaggtacatgtccagtgaaccaattatctttggagagtcgtctatctttgtagagtataagaaatttagcaacgataaaggctttcctaaagaatatggttctggtaagattgtgttatataacggcgttaattatctaaataatatctattgtttggaatatattaatacacataatgaagtgggtattaagtccgtggttgtacctattaagtttatagcagaattcttagttaatggagaaatacttaaacctagaattgataaaaccatgaaatatattaactcagaagattattatggaaatcaacataatatcatagtcgaacatttaagagatcaaagcatcaaaataggagatatctttaacgaggataaactatcggatgtgggacatcaatacgccaataatgataaatttagattaaatccagaagttagttattttacgaataaacgaactagaggaccgttgggaattttatcaaactacgtcaagactcttcttatttctatgtattgttccaaaacatttttagacgattccaacaaacgaaaggtattggcgattgattttggaaacggtgctgacctggaaaaatacttttatggagagattgcgttattggtagcgacggatccggatgctgatgctatagctagaggaaatgaaagatacaacaaattaaactctggaattaaaaccaagtactacaaatttgactacattcaggaaactattcgatccgatacatttgtctctagtgtcagagaagtattctattttggaaagtttaatatcatcgactggcagtttgctatccattattcttttcatccgagacattatgctaccgtcatgaataacttatccgaactaactgcttctggaggcaaggtattaatcactaccatggacggagacaaattatcaaaattaacagataaaaagacttttataattcataagaatttacctagtagcgaaaactatatgtctgtagaaaaaatagctgatgatagaatagtggtatataatccatcaacaatgtctactccaatgactgaatacattatcaaaaagaacgatatagtcagagtgtttaacgaatacggatttgttcttgtagataacgttgatttcgctacaattatagaacgaagtaaaaagtttattaatggcgcatctacaatggaagatagaccatctacaagaaactttttcgaactaaatagaggagccattaaatgtgaaggtttagatgtcgaagacttacttagttactatgttgtttatgtcttttctaagcggtaa

SEQ ID NO: 30 - DNA, 864 bp, Vaccinia virus
  source 1..864: mol_type = other DNA
atggatgaaattgtaaaaaatatccgggagggaacgcatgtccttcttccattttatgaaacattgccagaacttaatctgtctctaggtaaaagcccattacctagtctggaatacggagctaattactttcttcagatttctagagttaatgatctaaatagaatgccgaccgacatgttaaaactttttacacatgatatcatgttaccagaaagcgatctagataaagtctatgaaattttaaagattaatagcgtaaagtattatgggaggagtactaaagcggacgccgtagttgccgacctcagcgcacgcaataaactgttcaaacgtgaacgagatgctattaaatctaataatcatctcactgaaaacaatctatacattagcgattataagatgttaaccttcgacgtgtttcgaccattatttgattttgtaaacgaaaaatattgtattattaaacttccaactttattcggtagaggtgtaatcgatactatgagaatatattgtagtctctttaaaaatgttagactgctaaaatgcgtaagcgatagctggttaaaagatagcgccattatggtggctagtgatgtttgtaaaaaaaatttggatttatttatgtctcatgttaagtccgtcactaagtcttcttcttggaaggatgtgaacagtgttcaatttagtattttaaacaatccagtggatacggaattcattaataagttcttagagttttcgaatagagtatacgaagctctctattacgttcactcgttgctttattctagtatgacttctgattcaaaaagtatcgaaaacaaacatcagagaagactagttaaactactgctgtga

SEQ ID NO: 31 - DNA, 516 bp, Oplophorus gracilirostris
  source 1..516: mol_type = other DNA
atggtcttcacactcgaagatttcgttggggactggcgacagacagccggctacaacctggaccaagtccttgaacagggaggtgtgtccagtttgtttcagaatctcggggtgtccgtaactccgatccaaaggattgtcctgagcggtgaaaatgggctgaagatcgacatccatgtcatcatcccgtatgaaggtctgagcggcgaccaaatgggccagatcgaaaaaatttttaaggtggtgtaccctgtggatgatcatcactttaaggtgatcctgcactatggcacactggtaatcgacggggttacgccgaacatgatcgactatttcggacggccgtatgaaggcatcgccgtgttcgacggcaaaaagatcactgtaacagggaccctgtggaacggcaacaaaattatcgacgagcgcctgatcaaccccgacggctccctgctgttccgagtaaccatcaacggagtgaccggctggcggctgtgcgaacgcattctggcgtaa

SEQ ID NO: 32 - DNA, 750 bp, Rotavirus
  source 1..750: mol_type = other DNA
ggcttttaaaagttctgttccgagagagcgcgtgcggaaagatggataagcttgccgacctcaactacacattgagtgtaatcactctaatgaatgacacattgcattctataattcaggatcctggaatggcgtattttacatatattgcatctgttctaacagttttgttcacattacataaagcttcaattccaaccatgaaaatagcattgaaaacatcaaaatgttcatataaagtgattaaatattgtatagtcacgatcattaatactcttttaagattggctggatataaagagcaggttactactaaagacgaaattgagcaacagatggatagaattgttaaagagatgagacgtcagctggagatgattgataaactaactactcgtgaaattgaacaggttgaattgcttaaaagtatacatgacaacttgataactagatcagttgacgttatagatatgtcgaaggaattcaatcagaaaaacatcaaaacgctagatgaatgggagagtggaaggaatccatatgaaccgtcagaggtgactgcatccatgtgagaggttgagttaccgtcgtctgtcttcggaagcggcggaactcttcaccgcaagccccattagacctgatgattgactgagaagccacagtcaatcatatcgcgtgtggctcagccttaatcccgtttaaccaatccagcgagtgttggacgttaatggaaggaatggtcttagtgtgacc

SEQ ID NO: 33 - DNA, 696 bp, Zoanthus sp.
  source 1..696: mol_type = other DNA
atggctcagtcaaagcacggtctaacaaaagaaatgacaatgaaataccgtatggaagggtgcgtcgatggacataaatttgtgatcacgggagagggcattggatatccgttcaaagggaaacaggctattaatctgtgtgtggtcgaaggtggaccattgccatttgccgaagacatattgtcagctgcctttatgtacggaaacagggttttcactgaatatcctcaagacatagctgactatttcaagaactcgtgtcctgctggttatacatgggacaggtcttttctctttgaggatggagcagtttgcatatgtaatgcagatataacagtgagtgttgaagaaaactgcatgtatcatgagtccaaattttatggagtgaattttcctgctgatggacctgtgatgaaaaagatgacagataactgggagccatcctgcgagaagatcataccagtacctaagcaggggatattgaaaggggatgtctccatgtacctccttctgaaggatggtgggcgtttacggtgccaattcgacacagtttacaaagcaaagtctgtgccaagaaagatgccggactggcacttcatccagcataagctcacccgtgaagaccgcagcgatgctaagaatcagaaatggcatctgacagaacatgctattgcatccggatctgcattgccctga